European Patent Application EP 4 509 525 A1, published February 19, 2025. Title: 반감기가 향상된 융합단백질 플랫폼. Applicant: 주식회사 아이엠바이오로직스. The sequence listing filed with the application follows.

SEQUENCE LISTING (33 sequences)

SEQ ID NO: 1 - protein, 227 aa, synthetic construct
  REGION 1..227
DKTHTCPPCPAPELLGGPSVFLFPPKPKDTLMISRTPEVTCVVVDVSHEDPEVKFNWYVDGVEVHNAKTKPREEQYNSTYRVVSVLTVLHQDWLNGKEYKCKVSNKALPAPIEKTISKAKGQPREPQVYTLPPSRDELTKNQVSLTCLVKGFYPSDIAVEWESNGQPENNYKTTPPVLDSDGSFFLYSKLTVDKSRWQQGNVFSCSVMHEALHNHYTQKSLSLSPGK

SEQ ID NO: 2 - protein, 227 aa, synthetic construct
  REGION 1..227
DKTHTCPPCPAPEAAGGPSVFLFPPKPKDTLMISRTPEVTCVVVDVSHEDPEVKFNWYVDGVEVHNAKTKPREEQYNSTYRVVSVLTVLHQDWLNGKEYKCKVSNKALPAPIEKTISKAKGQPREPQVYTLPPSRDELTKNQVSLTCLVKGFYPSDIAVEWESNGQPENNYKTTPPVLDSDGSFFLYSKLTVDKSRWQQGNVFSCSVMHEALHNHYTQKSLSLSPGK

SEQ ID NO: 3 - protein, 229 aa, synthetic construct
  REGION 1..229
ESKYGPPCPPCPAPEFLGGPSVFLFPPKPKDTLMISRTPEVTCVVVDVSQEDPEVQFNWYVDGVEVHNAKTKPREEQFNSTYRVVSVLTVLHQDWLNGKEYKCKVSNKGLPSSIEKTISKAKGQPREPQVYTLPPSQEEMTKNQVSLTCLVKGFYPSDIAVEWESNGQPENNYKTTPPVLDSDGSFFLYSRLTVDKSRWQEGNVFSCSVMHEALHNHYTQKSLSLSLGK

SEQ ID NO: 4 - protein, 348 aa, synthetic construct
IAELPPKVSVFVPPRDGFFGNPRKSKLICQATGFSPRQIQVSWLREGKQVGSGVTTDQVQAEAKESGPTTYKVTSTLTIKESDWLSQSMFTCRVDHRGLTFQQNASSMCVPDQDTAIRVFAIPPSFASIFLTKSTKLTCLVTDLTTYDSVTISWTRQNGEAVKTHTNISESHPNATFSAVGEASICEDDWNSGERFTCTVTHTDLPSPLKQTISRPKGVALHRPDVYLLPPAREQLNLRESATITCLVTGFSPADVFVQWMQRGQPLSPEKYVTSAPMPEPQAPGRYFAHSILTVSEEEWNTGETYTCVVAHEALPNRVTERTVDKSTGKPTLYNVSLVMSDTAGTCY

SEQ ID NO: 5 - DNA, 1044 bp, synthetic construct
  source 1..1044: mol_type = other DNA
atcgcagagcttcccccgaaagtcagcgtatttgtacctcctagagatggttttttcgggaacccaaggaaatccaaactgatctgtcaagctaccggcttttccccccggcaaatacaagtatcatggctgagagagggtaagcaggtcggtagcggcgtaactactgaccaagttcaggcagaagcaaaggaatcagggcctacgacgtacaaggtgacatcaacactgacaataaaggaaagtgattggctgtcccagtccatgtttacgtgcagagtcgaccacagaggactcacatttcaacagaatgcgtcaagtatgtgcgtgccagaccaagatacagcaatcagagtattcgcaattccccctagcttcgcctcaatcttcctcacgaaatccactaagcttacgtgcctcgtgaccgacctgacgacgtacgatagtgttacaatatcctggactagacagaatggggaagcagtgaaaacgcatacgaacattagtgagagtcacccaaatgccactttcagtgctgtcggcgaggcgtctatctgtgaggatgattggaatagtggagaacgattcacctgcactgtgactcatactgatttgcccagcccgcttaagcaaactatctcccggcccaagggagttgccctccaccgacctgacgtatatcttttgccccctgccagggagcaactcaatctgcgcgaatctgcaaccattacgtgcttggtgacaggtttttcaccagctgatgtctttgtgcagtggatgcagagggggcaaccactcagtccagagaagtacgttacgtcagcgcccatgccagagccccaagctccaggacgctactttgcacactcaatattgacggtcagcgaggaggaatggaatactggagagacttacacctgtgttgtagctcacgaggctttgccgaatcgggtgaccgagaggacagtcgacaagtctacgggaaaaccaactctttataacgtttccctggtaatgtctgataccgcagggacatgctat

SEQ ID NO: 6 - protein, 236 aa, synthetic construct
QDTAIRVFAIPPSFASIFLTKSTKLTCLVTDLTTYDSVTISWTRQNGEAVKTHTNISESHPNATFSAVGEASICEDDWNSGERFTCTVTHTDLPSPLKQTISRPKGVALHRPDVYLLPPAREQLNLRESATITCLVTGFSPADVFVQWMQRGQPLSPEKYVTSAPMPEPQAPGRYFAHSILTVSEEEWNTGETYTCVVAHEALPNRVTERTVDKSTGKPTLYNVSLVMSDTAGTCY

SEQ ID NO: 7 - DNA, 708 bp, synthetic construct
  source 1..708: mol_type = other DNA
caagatacagcaatcagagtattcgcaattccccctagcttcgcctcaatcttcctcacgaaatccactaagcttacgtgcctcgtgaccgacctgacgacgtacgatagtgttacaatatcctggactagacagaatggggaagcagtgaaaacgcatacgaacattagtgagagtcacccaaatgccactttcagtgctgtcggcgaggcgtctatctgtgaggatgattggaatagtggagaacgattcacctgcactgtgactcatactgatttgcccagcccgcttaagcaaactatctcccggcccaagggagttgccctccaccgacctgacgtatatcttttgccccctgccagggagcaactcaatctgcgcgaatctgcaaccattacgtgcttggtgacaggtttttcaccagctgatgtctttgtgcagtggatgcagagggggcaaccactcagtccagagaagtacgttacgtcagcgcccatgccagagccccaagctccaggacgctactttgcacactcaatattgacggtcagcgaggaggaatggaatactggagagacttacacctgtgttgtagctcacgaggctttgccgaatcgggtgaccgagaggacagtcgacaagtctacgggaaaaccaactctttataacgtttccctggtaatgtctgataccgcagggacatgctat

SEQ ID NO: 8 - protein, 112 aa, synthetic construct
IAELPPKVSVFVPPRDGFFGNPRKSKLICQATGFSPRQIQVSWLREGKQVGSGVTTDQVQAEAKESGPTTYKVTSTLTIKESDWLSQSMFTCRVDHRGLTFQQNASSMCVPD

SEQ ID NO: 9 - DNA, 336 bp, synthetic construct
  source 1..336: mol_type = other DNA
atcgcagagcttcccccgaaagtcagcgtatttgtacctcctagagatggttttttcgggaacccaaggaaatccaaactgatctgtcaagctaccggcttttccccccggcaaatacaagtatcatggctgagagagggtaagcaggtcggtagcggcgtaactactgaccaagttcaggcagaagcaaaggaatcagggcctacgacgtacaaggtgacatcaacactgacaataaaggaaagtgattggctgtcccagtccatgtttacgtgcagagtcgaccacagaggactcacatttcaacagaatgcgtcaagtatgtgcgtgccagac

SEQ ID NO: 10 - protein, 106 aa, synthetic construct
QDTAIRVFAIPPSFASIFLTKSTKLTCLVTDLTTYDSVTISWTRQNGEAVKTHTNISESHPNATFSAVGEASICEDDWNSGERFTCTVTHTDLPSPLKQTISRPKG

SEQ ID NO: 11 - DNA, 318 bp, synthetic construct
  source 1..318: mol_type = other DNA
caagatacagcaatcagagtattcgcaattccccctagcttcgcctcaatcttcctcacgaaatccactaagcttacgtgcctcgtgaccgacctgacgacgtacgatagtgttacaatatcctggactagacagaatggggaagcagtgaaaacgcatacgaacattagtgagagtcacccaaatgccactttcagtgctgtcggcgaggcgtctatctgtgaggatgattggaatagtggagaacgattcacctgcactgtgactcatactgatttgcccagcccgcttaagcaaactatctcccggcccaaggga

SEQ ID NO: 12 - protein, 130 aa, synthetic construct
VALHRPDVYLLPPAREQLNLRESATITCLVTGFSPADVFVQWMQRGQPLSPEKYVTSAPMPEPQAPGRYFAHSILTVSEEEWNTGETYTCVVAHEALPNRVTERTVDKSTGKPTLYNVSLVMSDTAGTCY

SEQ ID NO: 13 - DNA, 390 bp, synthetic construct
  source 1..390: mol_type = other DNA
gttgccctccaccgacctgacgtatatcttttgccccctgccagggagcaactcaatctgcgcgaatctgcaaccattacgtgcttggtgacaggtttttcaccagctgatgtctttgtgcagtggatgcagagggggcaaccactcagtccagagaagtacgttacgtcagcgcccatgccagagccccaagctccaggacgctactttgcacactcaatattgacggtcagcgaggaggaatggaatactggagagacttacacctgtgttgtagctcacgaggctttgccgaatcgggtgaccgagaggacagtcgacaagtctacgggaaaaccaactctttataacgtttccctggtaatgtctgataccgcagggacatgctat

SEQ ID NO: 14 - protein, 137 aa, synthetic construct
QEDERIVLVDNKCKCARITSRIIRSSEDPNEDIVERNIRIIVPLNNRENISDPTSPLRTRFVYHLSDLCKKCDPTEVELDNQIVTATQSNICDEDSATETCYTYDRNKCYTAVVPLVYGGETKMVETALTPDACYPD

SEQ ID NO: 15 - DNA, 411 bp, synthetic construct
  source 1..411: mol_type = other DNA
caggaagatgaaagaatcgttctggtagacaataagtgtaagtgtgccagaatcaccagccgaatcatacgcagctcagaagaccctaacgaggatattgtggaacgcaatatccgcattatagtaccactcaacaacagggagaacatttcagaccccacatcaccccttcgcacgcggtttgtgtatcatttgagcgatctttgtaagaagtgtgatccaacagaagtcgaactcgataaccagattgtaacagccactcagtccaatatatgcgacgaggattctgccacggaaacatgctatacttatgaccgcaataagtgttatactgccgtcgtaccgttggtatatggaggggaaacgaagatggtcgagactgctttgacgccggatgcctgttatccggat

SEQ ID NO: 16 - protein, 38 aa, synthetic construct
RNTGRGGEEKKKEKEKEEQEERETKTPECPSHTQPLGV

SEQ ID NO: 17 - DNA, 114 bp, synthetic construct
  source 1..114: mol_type = other DNA
cgcaataccggcagaggaggcgaagagaaaaaaaaggaaaaggagaaagaagaacaagaggaacgagaaactaagactccggagtgcccttctcatacacaacccctgggggtt

SEQ ID NO: 18 - protein, 19 aa, synthetic construct
VPSTPPTPSPSTPPTPSPS

SEQ ID NO: 19 - DNA, 57 bp, synthetic construct
  source 1..57: mol_type = other DNA
gtcccctcaactccacctaccccatctccctcaactccacctaccccatctccctca

SEQ ID NO: 20 - protein, 15 aa, synthetic construct
GGGGSGGGGSGGGGS

SEQ ID NO: 21 - DNA, 45 bp, synthetic construct
  source 1..45: mol_type = other DNA
gggggaggcggcagtggaggaggggggtcaggaggtgggggttca

SEQ ID NO: 22 - protein, 427 aa, synthetic construct
NLVPMVATVGCGGSGGGGSGGGGSIQRTPKIQVYSRHPAENGKSNFLNCYVSGFHPSDIEVDLLKNGERIEKVEHSDLSFSKDWSFYLLYYTEFTPTEKDEYACRVNHVTLSQPKIVKWDRDMGGGGSGGGGSGGGGSGGGGSGSHSMRYFFTSVSRPGRGEPRFIAVGYVDDTQFVRFDSDAASQRMEPRAPWIEQEGPEYWDGETRKVKAHSQTHRVDLGTLRGCYNQSEAGSHTVQRMYGCDVGSDWRFLRGYHEYAYDGKDYIALKEDLRSWTAADMAAQTTKHKWEAAHVAEQLRAYLEGTCVEWLRRYLENGKETLQRTDAPKTHMTHHAVSDHEATLRCWALSFYPAEITLTWQRDGEDQTQDTELVETRPAGDGTFQKWAAVVVPSGQEQRYTCHVQHEGLPKPLTLRWGSDYKDDDDK

SEQ ID NO: 23 - DNA, 1282 bp, synthetic construct
  source 1..1282: mol_type = other DNA
aacctggtgcccatggtggccaccgtgggttgtggtggtagtggaggggggggatcaggtggtggagggagcatccagcggacacccaaaatccaagtttactcccggcacccggcagagaatgggaaatccaattttttgaattgctacgtgtctggtttccatccttcagatatagaggtggatttgctgaaaaacggcgaacgcatagaaaaagttgagcactccgatctctctttctcaaaagactggtctttttatctcttgtattataccgagttcaccccaacggaaaaggacgaatatgcctgccgagtcaatcacgtaacattgtctcagcctaaaattgtcaaatgggacagggatatggggggcggaggttctggagggggaggcagtggcggtggtggatccggtggcggtggatctggctcccactcaatgcggtacttcttcacgagcgtgtcacgcccaggtcggggggagcccagatttattgcagtcggatatgtggacgatactcagtttgtgcgattcgactctgacgccgcgtcccagagaatggaacccagagcgccttggattgaacaggagggcccagaatactgggatggcgagaccaggaaagtcaaagcgcacagtcagacacacagagtagatctcgggactctgcgcggatgttataaccaatctgaagcagggtctcacacggtccaaagaatgtatggctgcgatgtcgggtctgactggcgcttcttgcggggctatcatgagtatgcgtacgacggaaaagattatatcgcactcaaagaagatctccggtcctggactgccgcagacatggccgcccaaaccaccaagcacaagtgggaggcggctcatgttgcggaacagttgcgcgcctacctggaggggacctgtgtggagtggctccgcaggtatctggagaacggaaaagaaactctgcagcgaactgatgcccccaaaacgcatatgactcaccacgctgtctctgaccatgaagccaccctgaggtgctgggccctgagcttctaccctgcggagatcacactgacctggcagcgggatggggaggaccagacccaggacacggagctcgtggagaccaggcctgcaggggatggaaccttccagaagtgggcggctgtggtggtgccttctggacaggagcagagatacacctgccatgtgcagcatgagggtttgcccaagcccctcaccctgagatgggggagtcgactacaaagacgatgacgacaag

SEQ ID NO: 24 - protein, 427 aa, synthetic construct
NLVPMVATVGCGGSGGGGSGGGGSIQRTPKIQVYSRHPAENGKSNFLNCYVSGFHPSDIEVDLLKNGERIEKVEHSDLSFSKDWSFYLLYYTEFTPTEKDEYACRVNHVTLSQPKIVKWDRDMGGGGSGGGGSGGGGSGGGGSGSHSMRYFFTSVSRPGRGEPRFIAVGYVDDTQFVRFDSDAASQRMEPRAPWIEQEGPEYWDGETRKVKAHSQTHRVDLGTLRGCYNQSEAGSHTVQRMYGCDVGSDWRFLRGYHEYAYDGKDYIALKEDLRSWTAADMAAQTTKHKWEAAHVAEQLRAYLEGTCVEWLRRYLENGKETLQRTDSPKAHVTHHSRPEDKVTLRCWALGFYPADITLTWQLNGEELIQDMELVETRPAGDGTFQKWASVVVPLGKEQYYTCHVYHQGLPEPLTLRWEPDYKDDDDK

SEQ ID NO: 25 - DNA, 1281 bp, synthetic construct
  source 1..1281: mol_type = other DNA
aacctggtgcccatggtggccaccgtgggttgtggtggtagtggaggggggggatcaggtggtggagggagcatccagcggacacccaaaatccaagtttactcccggcacccggcagagaatgggaaatccaattttttgaattgctacgtgtctggtttccatccttcagatatagaggtggatttgctgaaaaacggcgaacgcatagaaaaagttgagcactccgatctctctttctcaaaagactggtctttttatctcttgtattataccgagttcaccccaacggaaaaggacgaatatgcctgccgagtcaatcacgtaacattgtctcagcctaaaattgtcaaatgggacagggatatggggggcggaggttctggagggggaggcagtggcggtggtggatccggtggcggtggatctggctcccactcaatgcggtacttcttcacgagcgtgtcacgcccaggtcggggggagcccagatttattgcagtcggatatgtggacgatactcagtttgtgcgattcgactctgacgccgcgtcccagagaatggaacccagagcgccttggattgaacaggagggcccagaatactgggatggcgagaccaggaaagtcaaagcgcacagtcagacacacagagtagatctcgggactctgcgcggatgttataaccaatctgaagcagggtctcacacggtccaaagaatgtatggctgcgatgtcgggtctgactggcgcttcttgcggggctatcatgagtatgcgtacgacggaaaagattatatcgcactcaaagaagatctccggtcctggactgccgcagacatggccgcccaaaccaccaagcacaagtgggaggcggctcatgttgcggaacagttgcgcgcctacctggaggggacctgtgtggagtggctccgcaggtatctggagaacggaaaagaaactctgcagcgaactgatagccctaaagcacacgtcactcatcactcaagaccggaggataaggtgacgcttagatgttgggcgcttggattttaccctgcggacatcacgctgacgtggcaattgaacggggaggagctgattcaggacatggagcttgtagagactagacccgcgggcgacggcactttccagaaatgggcatcagtggtagtgccgctcggtaaagaacagtattatacatgtcatgtttaccaccagggattgcctgagccactcacgcttcgatgggaaccagactacaaagacgatgacgacaag

SEQ ID NO: 26 - protein, 220 aa, synthetic construct
DIVMTQSPDSLAVSLGERATINCKSSQSVLNSSNNKNNLAWYQQQPGQPPKLLIYWASTRESGVPDRFSGSGSGTDFTLTISSLQAEDVAVYFCQQYYRTPWTFGQGTKVEIKRTVAAPSVFIFPPSDEQLKSGTASVVCLLNNFYPREAKVQWKVDNALQSGNSQESVTEQDSKDSTYSLSSTLTLSKADYEKHKVYACEVTHQGLSSPVTKSFNRGEC

SEQ ID NO: 27 - DNA, 660 bp, synthetic construct
  source 1..660: mol_type = other DNA
gacattgtgatgacacagagccccgatagcctggccgtgtctctgggagaaagagccaccatcaactgcaagagcagccagagcgtgctgaacagcagcaacaacaagaacaacctggcctggtatcagcagcagcctggccagcctcctaagctgctgatctactgggccagcaccagagaaagcggcgtgcccgatagattttctggcagcggctctggcaccgacttcaccctgacaattagctccctgcaggccgaggatgtggccgtgtacttctgccagcagtactacagaaccccttggacctttggccagggcaccaaggtggaaatcaagcgtacggtggcggcgccatctgtcttcatcttcccgccatctgatgagcagttgaaatctggaactgcctctgttgtgtgcctgctgaataacttctatcccagagaggccaaagtacagtggaaggtggataacgccctccaatcgggtaactcccaggagagtgtcacagagcaggacagcaaggacagcacctacagcctcagcagcaccctgacgctgagcaaagcagactacgagaaacacaaagtctacgcctgcgaagtcacccatcagggcctgagctcgcccgtcacaaagagcttcaacaggggagagtgt

SEQ ID NO: 28 - protein, 451 aa, synthetic construct
QVQLQQSGPGLLKPSQTLSLTCAISGDSVSSNRAAWNWIRQSPSRGLEWLGRTYYRSKWYNDYAVSVQGRITLIPDTSKNQFSLRLNSVTPEDTAVYYCASVRAVAPFDYWGQGVLVTVSSASTKGPSVFPLAPSSKSTSGGTAALGCLVKDYFPEPVTVSWNSGALTSGVHTFPAVLQSSGLYSLSSVVTVPSSSLGTQTYICNVNHKPSNTKVDKKVEPKSCDKTHTCPPCPAPELLGGPSVFLFPPKPKDTLMISRTPEVTCVVVDVSHEDPEVKFNWYVDGVEVHNAKTKPREEQYNSTYRVVSVLTVLHQDWLNGKEYKCKVSNKALPAPIEKTISKAKGQPREPQVYTLPPSRDELTKNQVSLTCLVKGFYPSDIAVEWESNGQPENNYKTTPPVLDSDGSFFLYSKLTVDKSRWQQGNVFSCSVMHEALHNHYTQKSLSLSPGK

SEQ ID NO: 29 - DNA, 1353 bp, synthetic construct
  source 1..1353: mol_type = other DNA
caagtccaattgcagcagagcgggcctggattgttgaagccatcacaaacgcttagtttgacatgcgctatatccggggacagtgtcagcagcaaccgagcggcatggaattggataagacagagtccatccaggggacttgagtggctcggacggacttattatcggagtaaatggtataatgactacgctgtgagcgttcaaggtagaataactcttatacctgatacgagcaaaaatcaattctcactgcgcttgaatagcgtcaccccagaggacaccgccgtatattactgcgcctcagtccgggccgttgcaccattcgattactggggtcaaggagtgcttgttacggtttcatctgctagcaccaagggcccatcggtcttccccctggcaccctcctccaagagcacctctgggggcacagcggccctgggctgcctggtcaaggactacttccccgaaccggtgacggtgtcgtggaactcaggcgccctgaccagcggcgtgcacaccttcccggctgtcctacagtcctcaggactctactccctcagcagcgtggtgaccgtgccctccagcagcttgggcacccagacctacatctgcaacgtgaatcacaagcccagcaacaccaaggtggacaagaaagttgagcccaaatcttgtgacaaaactcacacatgcccaccgtgcccagcacctgaactcctggggggaccgtcagtcttcctcttccccccaaaacccaaggacaccctcatgatctcccggacccctgaggtcacatgcgtggtggtggacgtgagccacgaagaccctgaggtcaagttcaactggtacgtggacggcgtggaggtgcataatgccaagacaaagccgcgggaggagcagtacaacagcacgtaccgtgtggtcagcgtcctcaccgtcctgcaccaggactggctgaatggcaaggagtacaagtgcaaggtctccaacaaagccctcccagcccccatcgagaaaaccatctccaaagccaaagggcagccccgagaaccacaggtgtacaccctgcccccatcccgggatgagctgaccaagaaccaggtcagcctgacctgcctggtcaaaggcttctatcccagcgacatcgccgtggagtgggagagcaatgggcagccggagaacaactacaagaccacgcctcccgtgctggactccgacggctccttcttcctctacagcaagctcaccgtggacaagagcaggtggcagcaggggaacgtcttctcatgctccgtgatgcatgaggctctgcacaaccactacacgcagaagagcctctccctgtctccgggtaaa

SEQ ID NO: 30 - protein, 224 aa, synthetic construct
QVQLQQSGPGLLKPSQTLSLTCAISGDSVSSNRAAWNWIRQSPSRGLEWLGRTYYRSKWYNDYAVSVQGRITLIPDTSKNQFSLRLNSVTPEDTAVYYCASVRAVAPFDYWGQGVLVTVSSASTKGPSVFPLAPSSKSTSGGTAALGCLVKDYFPEPVTVSWNSGALTSGVHTFPAVLQSSGLYSLSSVVTVPSSSLGTQTYICNVNHKPSNTKVDKKVEPKSC

SEQ ID NO: 31 - DNA, 672 bp, synthetic construct
  source 1..672: mol_type = other DNA
caagtccaattgcagcagagcgggcctggattgttgaagccatcacaaacgcttagtttgacatgcgctatatccggggacagtgtcagcagcaaccgagcggcatggaattggataagacagagtccatccaggggacttgagtggctcggacggacttattatcggagtaaatggtataatgactacgctgtgagcgttcaaggtagaataactcttatacctgatacgagcaaaaatcaattctcactgcgcttgaatagcgtcaccccagaggacaccgccgtatattactgcgcctcagtccgggccgttgcaccattcgattactggggtcaaggagtgcttgttacggtttcatctgctagcaccaagggcccatcggtcttccccctggcaccctcctccaagagcacctctgggggcacagcggccctgggctgcctggtcaaggactacttccccgaaccggtgacggtgtcgtggaactcaggcgccctgaccagcggcgtgcacaccttcccggctgtcctacagtcctcaggactctactccctcagcagcgtggtgaccgtgccctccagcagcttgggcacccagacctacatctgcaacgtgaatcacaagcccagcaacaccaaggtggacaagaaagttgagcccaaatcttgt

SEQ ID NO: 32 - protein, 165 aa, synthetic construct
APPRLICDSRVLERYLLEAKEAENITTGCAEHCSLNENITVPDTKVNFYAWKRMEVGQQAVEVWQGLALLSEAVLRGQALLVNSSQPWEPLQLHVDKAVSGLRSLTTLLRALGAQKEAISPPDAASAAPLRTITADTFRKLFRVYSNFLRGKLKLYTGEACRTGD

SEQ ID NO: 33 - DNA, 495 bp, synthetic construct
  source 1..495: mol_type = other DNA
gccccaccacgcctcatctgtgacagccgagtcctggagaggtacctcttggaggccaaggaggccgagaatatcacgacgggctgtgctgaacactgcagcttgaatgagaatatcactgtcccagacaccaaagttaatttctatgcctggaagaggatggaggtcgggcagcaggccgtagaagtctggcagggcctggccctgctgtcggaagctgtcctgcggggccaggccctgttggtcaactcttcccagccgtgggagcccctgcagctgcatgtggataaagccgtcagtggccttcgcagcctcaccactctgcttcgggctctgggagcccagaaggaagccatctcccctccagatgcggcctcagctgctccactccgaacaatcactgctgacactttccgcaaactcttccgagtctactccaatttcctccggggaaagctgaagctgtacacaggggaggcctgcaggacaggggac